European Patent Application EP 4 198 132 A1, published June 21, 2023. Title: A recombinant microorganism for producing L-glutamic acid and a method for producing L-glutamic acid using the same. Applicant: CJ CheilJedang Corporation. The sequence listing filed with the application follows.

SEQUENCE LISTING (32 sequences)

SEQ ID NO: 1 - protein, 374 aa, Unknown
  SbtA
MDFLSNFLTDFVGQLQSPTLAFLIGGMVIAALGTQLVIPEAISTIIVFMLLTKIGLTGGMAIRNSNLTEMLLPVAFSVILGILIVFIARFTLAKLPNVRTVDALATGGLFGAVSGSTMAAALTTLEESKISYEAWAGALYPFMDIPALVTAIVVANIYLNKRKRKSAAASIEESFSKQPVAAGDYGDQTDYPRTRQEYLSQQEPEDNRVKIWPIIEESLQGPALSAMLLGLALGIFTKPESVYEGFYDPLFRGLLSILMLIMGMEAWSRIGELRKVAQWYVVYSLIAPIVHGFIAFGLGMIAHYATGFSLGGVVVLAVIAASSSDISGPPTLRAGIPSANPSAYIGSSTAIGTPIAIGVCIPLFIGLAQTLGAG

SEQ ID NO: 2 - DNA, 1125 bp, Artificial Sequence
  codon optimized sbtA
atggattttctttctaatttcttgaccgacttcgtgggtcaactgcagtcacccactctggcgtttctgatcggcggtatggtaatcgccgctctgggaactcaattggttattcccgaagccatctcaacgattatcgttttcatgttgcttactaaaattggacttaccggaggtatggcgattcggaatagcaacctgaccgagatgcttttgcccgtggccttctccgtcattttgggaattttgatcgtatttatcgcgcgtttcactttggctaagctccccaatgtgcgcactgtggacgcccttgctacgggtggtctcttcggtgcggtgtcaggaagcacgatggccgccgccctgactacgcttgaggaatcaaaaatttcatatgaagcatgggcaggagctttgtacccttttatggatattccggccttggtcacggcaattgttgttgccaacatctatttgaataaacggaaacgtaaaagcgccgcagcatcaatcgaagagagcttctcgaagcagcccgtagcggctggcgactatggagatcagactgattatccacgtacccgtcaggaatacctctctcagcaagagccggaggacaatcgcgtcaaaatttggccaatcattgaagagtcgcttcaaggcccagccctttcagctatgttgttgggacttgcactgggtattttcacgaaacctgaatcggtgtatgagggattctacgatcctctttttcgcggactcctgtcgattctgatgctgattatgggcatggaagcctggagccgtatcggcgagcttcgtaaggtagctcagtggtatgtcgtttactctttgatcgctccgatcgtacacggatttatcgcttttggactgggtatgatcgcccattacgctacgggattcagcctcggtggagtggtcgttctggccgtaattgccgcatcttcttctgatatctctggcccacctaccctgcgtgccggcattccgagcgcaaatccgtcggcatatatcggtagctctactgcaatcggaacccccatcgcaatcggtgtgtgtattcctctcttcatcggtctcgcccagacgcttggcgcgggctaa

SEQ ID NO: 3 - DNA, 1125 bp, Unknown
  sbtA
atggattttttgtccaatttcttgacggacttcgtgggacaattgcagtccccaaccctagcctttctgattggggggatggttattgccgcccttggcacccaattggtaattccagaggcgatttctacgatcatcgtctttatgttgctcactaagattggcctaaccgggggcatggcaattcggaactccaacttgacggaaatgctcctacccgtggcattctctgtgatattgggaattcttattgtcttcatcgcccgttttaccctggctaaactgcctaacgtcagaaccgtggatgccctggccaccggcggcttgtttggggcagtcagtggctctacaatggctgccgccctcactacgttggaagaatcaaaaatttcctacgaagcctgggctggtgctctgtatccctttatggatattcctgccctggtaacggcgatcgtcgtagctaatatttatctcaataagagaaaacgtaagtctgctgctgctagtattgaggaatcgttcagcaagcaacccgttgccgccggggattatggcgaccaaacggattatcctcgtacccgccaagagtatttaagccagcaagaaccggaagataatcgggtcaaaatctggccaattatcgaagaaagtttacaaggccctgccctatcagccatgttgttaggtcttgccctgggcatatttaccaagccggaaagtgtctatgaaggtttttatgatcctctttttcgaggactactttccatcttgatgctgattatgggcatggaagcttggtccagaattggtgaactacgtaaagtagctcaatggtatgtggtctatagcctaatagctcccatagtgcacgggtttattgcctttggtcttggtatgattgcccactatgctacgggtttcagtctgggtggtgtggtagttttagcagttatcgccgcttctagctctgatatctccgggcctcctaccttgcgagcaggtatcccatctgccaacccctctgcctatatcggttcatccaccgccatcggtactcccattgccatcggcgtgtgcataccgcttttcattgggcttgcccagacccttggtgcaggttaa

SEQ ID NO: 4 - protein, 564 aa, Unknown
  BicA
MQITNKIHFRNLQGDLFGGVTAAVIALPMALAFGIASGAGATAGLWGAVIVGFFAALFGGTPTLISEPTGPMTVVQTAVIASLVAADPDNGLAMAFTVVMMAGLFQIAFGLLKLGKYVTMMPYTVISGFMSGIGIILVILQLAPFLGQASPKGGVIGTLQALPNLVSNVRPVETLLALMTVGIIWFMPSRWKKFAPPQLVALVLGTIISITLFGDLDIRRIGEIQAGLPALQLPVFQADQLQRMLIDAAVLGMLGCIDALLTSVVADSLTRTEHNSNKELVGQGIGNVMSGLFGGLGGAGATMGTVVNIQSGGRTALSGLIRAMVLLVVILGAAKLAATIPLAVLAGIAFKVGVDIIDWGFLKRAHHVSIKGALIMYAVIVLTVLVDLIAAVGIGVFIANILTIDRMSALQSKAVKSISDADDEILLSANEKRWLDEGNGRVLLFQLSGPMIFGVAKAIAREHNAIQECAAIVFDLSDVPHLGVTASLALENAIEEAAEKGRAVYIVGATGQTKRRLEKLQVFRFVPESNCYDDRSEALKDAVLALGPHESEDSPSSSSVQTTY

SEQ ID NO: 5 - DNA, 1695 bp, Artificial Sequence
  codon optimized bicA
atgcagattacgaacaagattcactttcgtaatttgcagggtgatctttttggcggcgttacggccgctgttattgcattgcctatggctttggcttttggaattgcatcgggtgcgggtgccacggccggactctggggagccgtaattgtgggcttcttcgccgcactgttcggaggaacccctacgcttatttcagagccaaccggacccatgaccgttgtgcagaccgccgtgatcgcttctcttgtagctgcggatcccgataacggccttgctatggcattcacggtggtgatgatggccggtttgtttcagattgccttcggtctgctcaaacttggaaaatatgtgaccatgatgccatatacggtaatctctggctttatgtccggcattggtattattttggtaattctgcaacttgcgcccttccttggacaagcttctccgaaaggaggcgtgatcggaacgctgcaagcacttcccaacctcgtgtcgaatgtacggcccgtagaaacgttgctggcattgatgaccgtcggtattatctggttcatgccttctcgttggaagaaattcgcgcctccgcaactcgtagccctggtactcggcacgattatttctatcacccttttcggagatcttgacattcgccggatcggagaaatccaagcgggcttgccagcccttcaactcccggttttccaagccgatcagttgcagcggatgctgatcgatgcagcagtcctcggaatgcttggatgtattgacgccctccttacgtcggtagttgccgattctctgacccgcaccgagcataactcgaataaagaactcgttggccaaggtatcggaaacgtaatgtcaggcttgttcggtggtctgggcggcgccggcgcaacgatgggcactgtggtgaacatccaatccggaggccgcacggccctgtctggtttgattcgcgctatggttctgctggtggtcatcttgggagctgcaaagctggcagccaccattccgcttgctgtgcttgctggaattgcgtttaaggtaggtgtagacattatcgactggggctttctgaagcgcgcacaccatgtgtcaattaagggcgcacttatcatgtatgctgttatcgtcctcactgtcctggtagatctcatcgccgcggttggtattggagtctttatcgcgaacattcttaccatcgaccggatgtcggccttgcaatcaaaagcggtgaaatcaatttctgatgcagatgacgaaattcttttgtctgccaatgaaaaacgttggttggacgaaggcaatggtcgcgtcttgctctttcagttgagcggacctatgatctttggagtggcaaaagcgatcgcacgggaacacaatgcgatccaggaatgtgctgccatcgtatttgacttgagcgacgttccccatctcggtgtcaccgcatcattggctcttgagaacgcaattgaagaggcagcagagaagggacgtgccgtttatatcgtgggcgccaccggacagaccaagcgccgtttggagaaacttcaagtctttcgcttcgtcccagaaagcaactgttacgacgaccgctctgaggcgcttaaagacgccgtgctcgcgttgggaccccatgagtcggaagattcgccgagcagctcttccgtgcagaccacttattga

SEQ ID NO: 6 - DNA, 1695 bp, Unknown
  bicA
atgcaaataactaacaaaattcattttaggaacctgcagggggacctttttggcggggttacagcggcggttattgccctgcccatggccttagccttcgggattgcttccggagcaggggctacggccggactctggggggcggtgatcgtagggtttttcgcggccttatttggcggcacccccaccttaatttccgaaccgactgggcccatgacggtggtgcaaacggcggttattgctagtttagtggcggcagatcccgacaatggcttggccatggccttcactgtggtaatgatggcggggttgttccagattgcctttggtctgctcaaattgggcaaatatgtcaccatgatgccctacacagtcatttccggctttatgtccggcattgggattattttggtgattttgcaactggctccctttcttggccaagctagtcccaagggaggggtaatcggcaccctccaggccctccctaacctagtaagcaatgtcaggccggtggaaaccctattggcgctcatgacggtgggcattatttggtttatgccttcccgttggaaaaagtttgctccgccccaattggtggctttagtgttggggacaattatttccatcaccctatttggcgatctggatatccgtcgcattggggaaattcaggccggtttgcccgctctacagctaccagtgtttcaggctgatcaattacagagaatgctgattgatgcggctgttctgggaatgctgggctgtattgatgccctcctgacttcggtggtggctgatagcttgacccgcacagaacataactccaacaaggaattagtcggccagggcatcggcaatgtaatgtccggtttatttggtggcttggggggagctggggccaccatggggacggtggtaaatatccagtccgggggacgcacagctctgtctggcttgatccgggcgatggtgttgctggtggtaattttaggcgcagctaaattggcggctaccattcccctagccgtattggctggtattgcgttcaaagttggggtggacattattgattgggggttcctcaagcgggctcaccatgtctccatcaaaggggccttgattatgtatgccgtcattgtcctgacggtgttggtggatttaattgcggcagtaggtattggtgtatttattgccaatattctcaccattgaccgtatgagtgcgttgcagtccaaagctgtgaaaagtattagcgatgccgacgacgaaattctcctttccgccaatgagaaacgttggctagatgagggcaatggccgggtcttgcttttccaactcagtggcccaatgatttttggggtggccaaggcgatcgccagggaacataatgccattcaagaatgtgccgccattgtttttgatctgagcgatgtgccccatttgggagtaaccgcttccctggccctggaaaatgccattgaagaagcggcggaaaaaggtcgggccgtttacattgtgggggcaacagggcaaaccaagcgacgcttggaaaaattgcaagtgttccgctttgttcctgaaagtaattgctatgacgaccgttctgaagctctcaaggacgctgtcctagctttgggacctcatgaaagtgaggactccccttccagttcttccgtccagaccacatactga

SEQ ID NO: 7 - DNA, 36 bp, Artificial Sequence
  CglE0286_up_F
aacgacggccagtgaattccggacgtttacgctgat

SEQ ID NO: 8 - DNA, 30 bp, Artificial Sequence
  CglE0286_up_R
agtactaaaccggaagggcctgtaaaggcc

SEQ ID NO: 9 - DNA, 37 bp, Artificial Sequence
  CglE0286_down_F
ccttccggtttagtactaaacaggaagagccccttta

SEQ ID NO: 10 - DNA, 36 bp, Artificial Sequence
  CglE0286_down_R
tgcatgcctgcaggtcgaccgcatgtggtggcaaaa

SEQ ID NO: 11 - DNA, 1477 bp, Artificial Sequence
  CJ7-sbtA
ggcccttccggtttagtagaaacatcccagcgctactaatagggagcgttgaccttccttccacggaccggtaatcggagtgcctaaaaccgcatgcggcttaggctccaagataggttctgcgcggccgggtaatgcatcttctttagcaacaagttgaggggtaggtgcaaataagaacgacatagaaatcgtctcctttctgtttttaatcaacatacaccaccacctaaaaattccccgaccagcaagttcacagtattcgggcacaatatcgttgccaaaatattgtttcggaatatcatgggatacgtacccaacgaaaggaaacactcatggattttctttctaatttcttgaccgacttcgtgggtcaactgcagtcacccactctggcgtttctgatcggcggtatggtaatcgccgctctgggaactcaattggttattcccgaagccatctcaacgattatcgttttcatgttgcttactaaaattggacttaccggaggtatggcgattcggaatagcaacctgaccgagatgcttttgcccgtggccttctccgtcattttgggaattttgatcgtatttatcgcgcgtttcactttggctaagctccccaatgtgcgcactgtggacgcccttgctacgggtggtctcttcggtgcggtgtcaggaagcacgatggccgccgccctgactacgcttgaggaatcaaaaatttcatatgaagcatgggcaggagctttgtacccttttatggatattccggccttggtcacggcaattgttgttgccaacatctatttgaataaacggaaacgtaaaagcgccgcagcatcaatcgaagagagcttctcgaagcagcccgtagcggctggcgactatggagatcagactgattatccacgtacccgtcaggaatacctctctcagcaagagccggaggacaatcgcgtcaaaatttggccaatcattgaagagtcgcttcaaggcccagccctttcagctatgttgttgggacttgcactgggtattttcacgaaacctgaatcggtgtatgagggattctacgatcctctttttcgcggactcctgtcgattctgatgctgattatgggcatggaagcctggagccgtatcggcgagcttcgtaaggtagctcagtggtatgtcgtttactctttgatcgctccgatcgtacacggatttatcgcttttggactgggtatgatcgcccattacgctacgggattcagcctcggtggagtggtcgttctggccgtaattgccgcatcttcttctgatatctctggcccacctaccctgcgtgccggcattccgagcgcaaatccgtcggcatatatcggtagctctactgcaatcggaacccccatcgcaatcggtgtgtgtattcctctcttcatcggtctcgcccagacgcttggcgcgggctaaactaaacaggaagagcc

SEQ ID NO: 12 - DNA, 17 bp, Artificial Sequence
  CJ7-sbtA_F
ggcccttccggtttagt

SEQ ID NO: 13 - DNA, 17 bp, Artificial Sequence
  CJ7-sbtA_R
ggctcttcctgtttagt

SEQ ID NO: 14 - DNA, 39 bp, Artificial Sequence
  CglE0085_up_F
aacgacggccagtgaattcgctcgaatgcctgactgaca

SEQ ID NO: 15 - DNA, 44 bp, Artificial Sequence
  CglE0085_up_R
gtttagtactaaaccggaagggccaaaggacgacttcacggtta

SEQ ID NO: 16 - DNA, 46 bp, Artificial Sequence
  CglE0085_down_F
ccggtttagtactaaacaggaagagccattgaggatgcgaaactgt

SEQ ID NO: 17 - DNA, 39 bp, Artificial Sequence
  CglE0085_down_R
tgcatgcctgcaggtcgacgtaatcgaatcaccggccag

SEQ ID NO: 18 - DNA, 2047 bp, Artificial Sequence
  CJ7-bicA
ggcccttccggtttagtagaaacatcccagcgctactaatagggagcgttgaccttccttccacggaccggtaatcggagtgcctaaaaccgcatgcggcttaggctccaagataggttctgcgcggccgggtaatgcatcttctttagcaacaagttgaggggtaggtgcaaataagaacgacatagaaatcgtctcctttctgtttttaatcaacatacaccaccacctaaaaattccccgaccagcaagttcacagtattcgggcacaatatcgttgccaaaatattgtttcggaatatcatgggatacgtacccaacgaaaggaaacactcatgcagattacgaacaagattcactttcgtaatttgcagggtgatctttttggcggcgttacggccgctgttattgcattgcctatggctttggcttttggaattgcatcgggtgcgggtgccacggccggactctggggagccgtaattgtgggcttcttcgccgcactgttcggaggaacccctacgcttatttcagagccaaccggacccatgaccgttgtgcagaccgccgtgatcgcttctcttgtagctgcggatcccgataacggccttgctatggcattcacggtggtgatgatggccggtttgtttcagattgccttcggtctgctcaaacttggaaaatatgtgaccatgatgccatatacggtaatctctggctttatgtccggcattggtattattttggtaattctgcaacttgcgcccttccttggacaagcttctccgaaaggaggcgtgatcggaacgctgcaagcacttcccaacctcgtgtcgaatgtacggcccgtagaaacgttgctggcattgatgaccgtcggtattatctggttcatgccttctcgttggaagaaattcgcgcctccgcaactcgtagccctggtactcggcacgattatttctatcacccttttcggagatcttgacattcgccggatcggagaaatccaagcgggcttgccagcccttcaactcccggttttccaagccgatcagttgcagcggatgctgatcgatgcagcagtcctcggaatgcttggatgtattgacgccctccttacgtcggtagttgccgattctctgacccgcaccgagcataactcgaataaagaactcgttggccaaggtatcggaaacgtaatgtcaggcttgttcggtggtctgggcggcgccggcgcaacgatgggcactgtggtgaacatccaatccggaggccgcacggccctgtctggtttgattcgcgctatggttctgctggtggtcatcttgggagctgcaaagctggcagccaccattccgcttgctgtgcttgctggaattgcgtttaaggtaggtgtagacattatcgactggggctttctgaagcgcgcacaccatgtgtcaattaagggcgcacttatcatgtatgctgttatcgtcctcactgtcctggtagatctcatcgccgcggttggtattggagtctttatcgcgaacattcttaccatcgaccggatgtcggccttgcaatcaaaagcggtgaaatcaatttctgatgcagatgacgaaattcttttgtctgccaatgaaaaacgttggttggacgaaggcaatggtcgcgtcttgctctttcagttgagcggacctatgatctttggagtggcaaaagcgatcgcacgggaacacaatgcgatccaggaatgtgctgccatcgtatttgacttgagcgacgttccccatctcggtgtcaccgcatcattggctcttgagaacgcaattgaagaggcagcagagaagggacgtgccgtttatatcgtgggcgccaccggacagaccaagcgccgtttggagaaacttcaagtctttcgcttcgtcccagaaagcaactgttacgacgaccgctctgaggcgcttaaagacgccgtgctcgcgttgggaccccatgagtcggaagattcgccgagcagctcttccgtgcagaccacttattgaactaaacaggaagagcc

SEQ ID NO: 19 - DNA, 38 bp, Artificial Sequence
  odhA_up_F
tgaattcgagctcggtacccttgaacggaattgggtgg

SEQ ID NO: 20 - DNA, 38 bp, Artificial Sequence
  odhA_up_R
cccaggtggcatcggtaccttcacccagcgccacgcag

SEQ ID NO: 21 - DNA, 39 bp, Artificial Sequence
  odhA_down_F
cgctgggtgaaggtaccgatgccacctgggttggtcaag

SEQ ID NO: 22 - DNA, 38 bp, Artificial Sequence
  odhA_down_R
gtcgactctagaggatccccggacaaggaatggagaga

SEQ ID NO: 23 - DNA, 18 bp, Artificial Sequence
  odhA_del_F
cttaccgttgttgccctt

SEQ ID NO: 24 - DNA, 19 bp, Artificial Sequence
  odhA_del_R
ctccttcacccacatcatt

SEQ ID NO: 25 - DNA, 19 bp, Artificial Sequence
  CJ7-sbtA_confirm_F
caagcagcaagtgccacac

SEQ ID NO: 26 - DNA, 18 bp, Artificial Sequence
  CJ7-sbtA_confirm_R
ccaactgctccgacgaag

SEQ ID NO: 27 - DNA, 18 bp, Artificial Sequence
  CJ7-bicA_confirm_F
attcccaaaggtgccagc

SEQ ID NO: 28 - DNA, 18 bp, Artificial Sequence
  CJ7-bicA_confirm_R
cagtgcgcaaaaggcctc

SEQ ID NO: 29 - protein, 1221 aa, Unknown
  OdhA
MSSASTFGQNAWLVDEMFQQFQKDPKSVDKEWRELFEAQGGPNATPATTEAQPSAPKESAKPAPKAAPAAKAAPRVETKPAAKTAPKAKESSVPQQPKLPEPGQTPIRGIFKSIAKNMDISLEIPTATSVRDMPARLMFENRAMVNDQLKRTRGGKISFTHIIGYAMVKAVMAHPDMNNSYDVIDGKPTLIVPEHINLGLAIDLPQKDGSRALVVAAIKETEKMNFSEFLAAYEDIVTRSRKGKLTMDDYQGVTVSLTNPGGIGTRHSVPRLTKGQGTIIGVGSMDYPAEFQGASEDRLAELGVGKLVTITSTYDHRVIQGAVSGEFLRTMSRLLTDDSFWDEIFDAMNVPYTPMRWAQDVPNTGVDKNTRVMQLIEAYRSRGHLIADTNPLSWVQPGMPVPDHRDLDIETHSLTIWDLDRTFSVGGFGGKETMTLREVLSRLRAAYTLKVGSEYTHILDRDERTWLQDRLEAGMPKPTQAEQKYILQKLNAAEAFENFLQTKYVGQKRFSLEGAEALIPLMDSAIDTAAGQGLDEVVIGMPHRGRLNVLFNIVGKPLASIFNEFEGQMEQGQIGGSGDVKYHLGSEGQHLQMFGDGEIKVSLTANPSHLEAVNPVMEGIVRAKQDYLDKGVDGKTVVPLLLHGDAAFAGLGIVPETINLAKLRGYDVGGTIHIVVNNQIGFTTTPDSSRSMHYATDYAKAFGCPVFHVNGDDPEAVVWVGQLATEYRRRFGKDVFIDLVCYRLRGHNEADDPSMTQPKMYELITGRETVRAQYTEDLLGRGDLSNEDAEAVVRDFHDQMESVFNEVKEGGKKQAEAQTGITGSQKLPHGLETNISREELLELGQAFANTPEGFNYHPRVAPVAKKRVSSVTEGGIDWAWGELLAFGSLANSGRLVRLAGEDSRRGTFTQRHAVAIDPATAEEFNPLHELAQSKGNNGKFLVYNSALTEYAGMGFEYGYSVGNEDSVVAWEAQFGDFANGAQTIIDEYVSSGEAKWGQTSKLILLLPHGYEGQGPDHSSARIERFLQLCAEGSMTVAQPSTPANHFHLLRRHALSDLKRPLVIFTPKSMLRNKAAASAPEDFTEVTKFQSVIDDPNVADAAKVKKVMLVSGKLYYELAKRKEKDGRDDIAIVRIEMLHPIPFNRISEALAGYPNAEEVLFVQDEPANQGPWPFYQEHLPELIPNMPKMRRVSRRAQSSTATGVAKVHQLEEKQLIDEAFEA

SEQ ID NO: 30 - protein, 373 aa, Unknown
  SbtA
MDFLSHFLTDFVGQLQSPTLAFLIGGMVIAALGTQLVIPEAISTIIVFMLLTKIGLTGGMAIRNSNLTEMLLPMIFSVILGILIVFIARFTLAKLPNVKTVDALATGGLFGAVSGSTMAAALTTLEESKISYEAWAGALYPFMDIPALVTAIVVANIYLNKKKRRAAAAIEGSLSKQPVAAGDYGDQQDYPRTRQEYLSQQEPEDNRVKIWPIIEESLQGPALSAMLLGLALGIFTKPESVYEGFYDPLFRGLLSILMLIMGMEAWSRIGELRKVAQWYVVYSLVAPIVHGFIAFGLGMIAHYTTGFSLGGVVVLAVIAASSSDISGPPTLRAGIPSANPSAYIGASTAIGTPIAIGVCIPLFIGLAQTLGAG

SEQ ID NO: 31 - DNA, 1119 bp, Unknown
  SbtA
atggattttttatcccactttttaacggattttgttggacagttgcagtccccaaccctagcctttttgattggggggatggttattgccgcccttggtacccaattggtaattccagaggcgatttctacgatcatcgtctttatgttgctcactaagattggcctgaccgggggcatggcaattcgcaactccaacttaacggaaatgctcctgccgatgatattctccgtaatattgggaattctaattgtattcatcgcccgttttaccctggctaaacttcccaatgttaaaaccgtggatgcccttgccactggtggcttgtttggggcagttagtggttctacgatggccgccgccctaactacgttggaagaatcaaaaatttcctacgaagcttgggctggtgccctctatccttttatggatattcctgccctagtaacggcgatcgtagtggccaatatttatctcaataagaagaagcgtcgtgccgcggccgccattgagggatctttaagcaagcaacccgttgccgcaggggattatggcgatcagcaggattatcctcgtacccgccaggagtatttgagccagcaggaaccggaggataatcgggtcaagatctggccgatcatcgaagaaagtttacaaggtcccgccctgtcagccatgttattaggtcttgcccttggcatatttaccaagccggaaagtgtctatgaaggtttctatgatcctctttttcgaggcctactttctatcttgatgctcattatggggatggaggcttggtccagaattggcgaactacgtaaagtagctcaatggtatgtggtctatagcctggtagctccgatagtgcacgggtttattgcctttggtcttggtatgattgcccactacactacgggattcagcctgggcggtgtcgtagttttagcagtcatcgccgcttctagttctgatatctccggcccccccaccttgcgagccggtatcccgtcggccaatccctctgcttatattggtgcatccaccgctatcggtactcccattgccatcggcgtgtgcataccgcttttcattgggcttgcccagacccttggtgcaggt

SEQ ID NO: 32 - DNA, 5803 bp, Artificial Sequence
  pDCM2
gttcgcttgctgtccataaaaccgcccagtctagctatcgccatgtaagcccactgcaagctacctgctttctctttgcgcttgcgttttcccttgtccagatagcccagtagctgacattcatccggggtcagcaccgtttctgcggactggctttctacgtgttccgcttcctttagcagcccttgcgccctgagtgcttgcggcagcgtgaagctagcttttatcgccattcgccattcaggctgcgcaactgttgggaagggcgatcggtgcgggcctcttcgctattacgccagctggcgaaagggggatgtgctgcaaggcgattaagttgggtaacgccagggttttcccagtcacgacgttgtaaaacgacggccagtgaattcgagctcggtacccggggatcctctagagtcgacctgcaggcatgcaagcttggcgtaatcatggtcatagctgtttcctgtgtgaaattgttatccgctcacaattccacacaacatacgagccggaagcataaagtgtaaagcctggggtgcctaatgagtgagctaactcacattaattgcgttgcgctcactgcccgctttccagtcgggaaacctgtcgtgccagctgcattaatgaatcggccaacgcgcggggagaggcggtttgcgtattgggcgctcttccgcttcctcgctcactgactcgctgcgctcggtcgttcggctgcggcgagcggtatcagctcactcaaaggcggtaatacggttatccacagaatcaggggataacgcaggaaagaacatgtgagcaaaaggccagcaaaaggccaggaaccgtaaaaaggccgcgttgctggcgtttttccataggctccgcccccctgacgagcatcacaaaaatcgacgctcaagtcagaggtggcgaaacccgacaggactataaagataccaggcgtttccccctggaagctccctcgtgcgctctcctgttccgaccctgccgcttaccggatacctgtccgcctttctcccttcgggaagcgtggcgctttctcaatgctcacgctgtaggtatctcagttcggtgtaggtcgttcgctccaagctgggctgtgtgcacgaaccccccgttcagcccgaccgctgcgccttatccggtaactatcgtcttgagtccaacccggtaagacacgacttatcgccactggcagcagccactggtaacaggattagcagagcgaggtatgtaggcggtgctacagagttcttgaagtggtggcctaactacggctacactagaaggacagtatttggtatctgcgctctgctgaagccagttaccttcggaaaaagagttggtagctcttgatccggcaaacaaaccaccgctggtagcggtggtttttttgtttgcaagcagcagattacgcgcagaaaaaaaggatctcaagaagatcctttgatcttttctacggggtctgacgctcagtggaacgaaaactcacgttaagggattttggtcatgagattatcaaaaaggatcttcacctagatccttttggggtgggcgaagaactccagcatgagatccccgcgctggaggatcatccagccctgatagaaacagaagccactggagcacctcaaaaacaccatcatacactaaatcagtaagttggcagcatcacccgacgcactttgcgccgaataaatacctgtgacggaagatcacttcgcagaataaataaatcctggtgtccctgttgataccgggaagccctgggccaacttttggcgaaaatgagacgttgatcggcacgtaagaggttccaactttcaccataatgaaataagatcactaccgggcgtattttttgagttatcgagattttcaggagctgatagaaacagaagccactggagcacctcaaaaacaccatcatacactaaatcagtaagttggcagcatcacccgacgcactttgcgccgaataaatacctgtgacggaagatcacttcgcagaataaataaatcctggtgtccctgttgataccgggaagccctgggccaacttttggcgaaaatgagacgttgatcggcacgtaagaggttccaactttcaccataatgaaataagatcactaccgggcgtattttttgagttatcgagattttcaggagctctttggcatcgtctctcgcctgtcccctcagttcagtaatttcctgcatttgcctgtttccagtcggtagatattccacaaaacagcagggaagcagcgcttttccgctgcataaccctgcttcggggtcattatagcgattttttcggtatatccatcctttttcgcacgatatacaggattttgccaaagggttcgtgtagactttccttggtgtatccaacggcgtcagccgggcaggataggtgaagtaggcccacccgcgagcgggtgttccttcttcactgtcccttattcgcacctggcggtgctcaacgggaatcctgctctgcgaggctggccggctaccgccggcgtaacagatgagggcaagcggatggctgatgaaaccaagccaaccaggaagggcagcccacctatcaaggtgtactgccttccagacgaacgaagagcgattgaggaaaaggcggcggcggccggcatgagcctgtcggcctacctgctggccgtcggccagggctacaaaatcacgggcgtcgtggactatgagcacgtccgcgagggcgtcccggaaaacgattccgaagcccaacctttcatagaaggcggcggtggaatcgaaatctcgtgatggcaggttgggcgtcgcttggtcggtcatttcgaaaaaggttaggaatacggttagccatttgcctgcttttatatagttcantatgggattcacctttatgttgataagaaataaaagaaaatgccaataggatatcggcattttcttttgcgtttttatttgttaactgttaattgtccttgttcaaggatgctgtctttgacaacagatgttttcttgcctttgatgttcagcaggaagctcggcgcaaacgttgattgtttgtctgcgtagaatcctctgtttgtcatatagcttgtaatcacgacattgtttcctttcgcttgaggtacagcgaagtgtgagtaagtaaaggttacatcgttaggcggatcaagatccatttttaacacaaggccagttttgttcagcggcttgtatgggccagttaaagaattagaaacataaccaagcatgtaaatatcgttagacgtaatgccgtcaatcgtcatttttgatccgcgggagtcagtgaacaggtaccatttgccgttcattttaaagacgttcgcgcgttcaatttcatctgttactgtgttagatgcaatcagcggtttcatcacttttttcagtgtgtaatcatcgtttagctcaatcataccgagagcgccgtttgctaactcagccgtgcgttttttatcgctttgcagaagtttttgactttcttgacggaagaatgatgtgcttttgccatagtatgctttgttaaataaagattcttcgccttggtagccatcttcagttccagtgtttgcttcaaatactaagtatttgtggcctttatcttctacgtagtgaggatctctcagcgtatggttgtcgcctgagctgtagttgccttcatcgatgaactgctgtacattttgatacgtttttccgtcaccgtcaaagattgatttataatcctctacaccgttgatgttcaaagagctgtctgatgctgatacgttaacttgtgcagttgtcagtgtttgtttgccgtaatgtttaccggagaaatcagtgtagaataaacggatttttccgtcagatgtaaatgtggctgaacctgaccattcttgtgtttggtcttttaggatagaatcatttgcatcgaatttgtcgctgtctttaaagacgcggccagcgtttttccagctgtcaatagaagtttcgccgactttttgatagaacatgtaaatcgatgtgtcatccgcatttttaggatctccggctaatgcaaagacgatgtggtagccgtgatagtttgcgacagtgccgtcagcgttttgtaatggccagctgtcccaaacgtccaggccttttgcagaagagatatttttaattgtggacgaatcaaattcagaaacttgatatttttcatttttttgctgttcagggatttgcagcatatcatggcgtgtaatatgggaaatgccgtatgtttccttatatggcttttggttcgtttctttcgcaaacgcttgagttgcgcctcctgccagcagtgcggtagtaaaggttaatactgttgcttgttttgcaaactttttgatgttcatcgttcatgtctccttttttatgtactgtgttagcggtctgcttcttccagccctcctgtttgaagatggcaagttagttacgcacaataaaaaaagacctaaaatatgtaaggggtgacgccaaagtatacactttgccctttacacattttaggtcttgcctgctttatcagtaacaaacccgcgcgatttacttttcgacctcattctattagactctcgtttggattgcaactggtctattttcctcttttgtttgatagaaaatcataaaaggatttgcagactacgggcctaaagaactaaaaaatctatctgtttcttttcattctctgtattttttatagtttctgttgcatgggcataaagttgcctttttaatcacaattcagaaaatatcataatatctcatttcactaaataatagtgaacggcaggtatatgtgatgggttaaaaaggatcaccccagagtcccgctcagaagaactcgtcaagaaggcgatagaaggcgatgcgctgcgaatcgggagcggcgataccgtaaagcacgaggaagcggtcagcccattcgccgccaagctcttcagcaatatcacgggtagccaacgctatgtcctgatagcggtccgccacacccagccggccacagtcgatgaatccagaaaagcggccattttccaccatgatattcggcaagcaggcatcgccatgggtcacgacgagatcctcgccgtcgggcatccgcgccttgagcctggcgaacagttcggctggcgcgagcccctgatgctcttcgtccagatcatcctgatcgacaagaccggcttccatccgagtacgtgctcgctcgatgcgatgtttcgcttggtggtcgaatgggcaggtagccggatcaagcgtatgcagccgccgcattgcatcagccatgatggatactttctcggcaggagcaaggtgagatgacaggagatcctgccccggcacttcgcccaatagcagccagtcccttcccgcttcagtgacaacgtcgagacagctgcgcaaggaacgcccgtcgtggccagccacgatagccgcgctgcctcgtcttggagttcattcagggcaccggacaggtcggtcttgacaaaaagaaccgggcgcccctgcgctgacagccggaacacggcggcatcagagcagccgattgtctgttgtgcccagtcatagccgaatagcctctccacccaagcggccggagaacctgcgtgcaatccatcttgttcaatcatgcgaaacgatcctcatcctgtctcttgatcagatcttgatcccctgcgccatcagatccttggcggcaagaaagccatccagtttactttgcagggcttcccaaccttaccagagggcgccccagctggcaattccg